European Patent Application EP 4 400 518 A1, published July 17, 2024. Title: 抗原靶向、抗CD16A和免疫效应细胞激活三功能融合蛋白及其应用. Applicant: 启愈生物技术（上海）有限公司. The sequence listing filed with the application follows.

SEQUENCE LISTING (112 sequences)

SEQ ID NO: 1 - protein, 257 aa, synthetic construct
MDMRVPAQLLGLLLLWFPGSRCSYVLTQPSSVSVAPGQTATISCGGHNIGSKNVHWYQQRPGQSPVLVIYQDNKRPSGIPERFSGSNSGNTATLTISGTQAMDEADYYCQVWDNYSVLFGGGTKLTVLGGGGSGGGGSGGGGSNWVNVISDLKKIEDLIQSMHIDATLYTESDVHPSCKVTAMKCFLLELQVISCESGDASIHDTVENLIILANNSLSSNGNVTESGCKECEELEEKNIKEFLQSFVHIVQMFINTS

SEQ ID NO: 2 - protein, 456 aa, synthetic construct
MEFGLSWLFLVAILKGVQCQVQLVQSGAEVKKPGESLKVSCKASGYTFTSYYMHWVRQAPGQGLEWMGIINPSGGSTSYAQKFQGRVTMTRDTSTSTVYMELSSLRSEDTAVYYCARGSAYYYDFADYWGQGTLVTVSSGGGGSGGGGSGGGGSITCPPPMSVEHADIWVKSYSLYSRERYICNSGFKRKAGTCSLTECVLNKATNVAHWTTPSLKCIRGGGGSEPKSSDKTHTCPPCPAPELLGGPSVFLFPPKPKDTLMISRTPEVTCVVVDVSHEDPEVKFNWYVDGVEVHNAKTKPREEQYNSTYRVVSVLTVLHQDWLNGKEYKCKVSNKALPAPIEKTISKAKGQPREPQVYTLPPSRDELTKNQVSLWCLVKGFYPSDIAVEWESNGQPENNYKTTPPVLDSDGSFFLYSKLTVDKSRWQQGNVFSCSVMHEALHNHYTQKSLSLSPGK

SEQ ID NO: 3 - protein, 242 aa, synthetic construct
MDMRVPAQLLGLLLLWFPGSRCDIVMTQSPDSLTVSLGERTTINCKSSQSVLDSSTNKNSLAWYQQKPGQPPKLLLSWASTRESGIPDRFSGSGSGTDFTLTIDSPQPEDSATYYCQQSAHFPITFGQGTRLEIKRTVAAPSVFIFPPSDEQLKSGTASVVCLLNNFYPREAKVQWKVDNALQSGNSQESVTEQDSKDSTYSLSSTLTLSKADYEKHKVYACEVTHQGLSSPVTKSFNRGEC

SEQ ID NO: 4 - protein, 471 aa, synthetic construct
MEFGLSWLFLVAILKGVQCQVQLVQSGAEVKKPGESVKVSCKASGYTFTNYGMNWVKQAPGQGLEWMGWINTYTGEPTYADKFQGRVTMTTDTSTSTAYMEIRNLGGDDTAVYYCARWSWSDGYYVYFDYWGQGTSVTVSSASTKGPSVFPLAPSSKSTSGGTAALGCLVKDYFPEPVTVSWNSGALTSGVHTFPAVLQSSGLYSLSSVVTVPSSSLGTQTYICNVNHKPSNTKVDKKVEPKSCDKTHTCPPCPAPELLGGPSVFLFPPKPKDTLMISRTPEVTCVVVDVSHEDPEVKFNWYVDGVEVHNAKTKPREEQYNSTYRVVSVLTVLHQDWLNGKEYKCKVSNKALPAPIEKTISKAKGQPREPQVYTLPPSREEMTKNQVSLSCAVKGFYPSDIAVEWESNGQPENNYKTTPPVLDSDGSFFLVSKLTVDKSRWQQGNVFSCSVMHEALHNRYTQKSLSLSPGK

SEQ ID NO: 5 - protein, 456 aa, synthetic construct
MEFGLSWLFLVAILKGVQCQVQLVQSGAEVKKPGESLKVSCKASGYTFTSYYMHWVRQAPGQGLEWMGIINPSGGSTSYAQKFQGRVTMTRDTSTSTVYMELSSLRSEDTAVYYCARGSAYYYDFADYWGQGTLVTVSSGGGGSGGGGSGGGGSITCPPPMSVEHADIWVKSYSLYSRERYICNSGFKRKAGTCSLTECVLNKATNVAHWTTPSLKCIRGGGGSEPKSSDKTHTCPPCPAPEAAGGPSVFLFPPKPKDTLMISRTPEVTCVVVDVSHEDPEVKFNWYVDGVEVHNAKTKPREEQYNSTYRVVSVLTVLHQDWLNGKEYKCKVSNKALPAPIEKTISKAKGQPREPQVYTLPPSRDELTKNQVSLWCLVKGFYPSDIAVEWESNGQPENNYKTTPPVLDSDGSFFLYSKLTVDKSRWQQGNVFSCSVMHEALHNHYTQKSLSLSPGK

SEQ ID NO: 6 - protein, 471 aa, synthetic construct
MEFGLSWLFLVAILKGVQCQVQLVQSGAEVKKPGESVKVSCKASGYTFTNYGMNWVKQAPGQGLEWMGWINTYTGEPTYADKFQGRVTMTTDTSTSTAYMEIRNLGGDDTAVYYCARWSWSDGYYVYFDYWGQGTSVTVSSASTKGPSVFPLAPSSKSTSGGTAALGCLVKDYFPEPVTVSWNSGALTSGVHTFPAVLQSSGLYSLSSVVTVPSSSLGTQTYICNVNHKPSNTKVDKKVEPKSCDKTHTCPPCPAPEAAGGPSVFLFPPKPKDTLMISRTPEVTCVVVDVSHEDPEVKFNWYVDGVEVHNAKTKPREEQYNSTYRVVSVLTVLHQDWLNGKEYKCKVSNKALPAPIEKTISKAKGQPREPQVYTLPPSREEMTKNQVSLSCAVKGFYPSDIAVEWESNGQPENNYKTTPPVLDSDGSFFLVSKLTVDKSRWQQGNVFSCSVMHEALHNRYTQKSLSLSPGK

SEQ ID NO: 7 - protein, 213 aa, synthetic construct
SYVLTQPSSVSVAPGQTATISCGGHNIGSKNVHWYQQRPGQSPVLVIYQDNKRPSGIPERFSGSNSGNTATLTISGTQAMDEADYYCQVWDNYSVLFGGGTKLTVLRTVAAPSVFIFPPSDEQLKSGTASVVCLLNNFYPREAKVQWKVDNALQSGNSQESVTEQDSKDSTYSLSSTLTLSKADYEKHKVYACEVTHQGLSSPVTKSFNRGEC

SEQ ID NO: 8 - protein, 478 aa, synthetic construct
MEFGLSWLFLVAILKGVQCQVQLVQSGAEVKKPGESLKVSCKASGYTFTSYYMHWVRQAPGQGLEWMGIINPSGGSTSYAQKFQGRVTMTRDTSTSTVYMELSSLRSEDTAVYYCARGSAYYYDFADYWGQGTLVTVSSASTKGPSVFPLAPSSKSTSGGTAALGCLVKDYFPEPVTVSWNSGALTSGVHTFPAVLQSSGLYSLSSVVTVPSSSLGTQTYICNVNHKPSNTKVDKKVEPKSCDKTHTCPPCPAPEAAGGPSVFLFPPKPKDTLMISRTPEVTCVVVDVSHEDPEVKFNWYVDGVEVHNAKTKPREEQYNSTYRVVSVLTVLHQDWLNGKEYKCKVSNKALPAPIEKTISKAKGQPREPQVYTLPPSREEMTKNQVSLSCAVKGFYPSDIAVEWESNGQPENNYKTTPPVLDSDGSFFLVSKLTVDKSRWQQGNVFSCSVMHEALHNRYTQKSLSLSPGKGGSHHHHHH

SEQ ID NO: 9 - protein, 469 aa, synthetic construct
MEFGLSWLFLVAILKGVQCQVQLVQSGAEVKKPGESVKVSCKASGYTFTNYGMNWVKQAPGQGLEWMGWINTYTGEPTYADKFQGRVTMTTDTSTSTAYMEIRNLGGDDTAVYYCARWSWSDGYYVYFDYWGQGTSVTVSSGGGGSGGGGSGGGGSITCPPPMSVEHADIWVKSYSLYSRERYICNSGFKRKAGTCSLTECVLNKATNVAHWTTPSLKCIRGGGGSEPKSSDKTHTCPPCPAPEAAGGPSVFLFPPKPKDTLMISRTPEVTCVVVDVSHEDPEVKFNWYVDGVEVHNAKTKPREEQYNSTYRVVSVLTVLHQDWLNGKEYKCKVSNKALPAPIEKTISKAKGQPREPQVYTLPPSRDELTKNQVSLWCLVKGFYPSDIAVEWESNGQPENNYKTTPPVLDSDGSFFLYSKLTVDKSRWQQGNVFSCSVMHEALHNHYTQKSLSLSPGKGGSDYKDDDDK

SEQ ID NO: 10 - protein, 242 aa, synthetic construct
DIVMTQSPDSLTVSLGERTTINCKSSQSVLDSSTNKNSLAWYQQKPGQPPKLLLSWASTRESGIPDRFSGSGSGTDFTLTIDSPQPEDSATYYCQQSAHFPITFGQGTRLEIKGGGGSGGGGSGGGGSNWVNVISDLKKIEDLIQSMHIDATLYTESDVHPSCKVTAMKCFLLELQVISCESGDASIHDTVENLIILANNSLSSNGNVTESGCKECEELEEKNIKEFLQSFVHIVQMFINTS

SEQ ID NO: 11 - protein, 236 aa, synthetic construct
MDMRVPAQLLGLLLLWFPGSRCEIVLTQSPATLSLSPGERATLSCRASQSVSSYLAWYQQKPGQAPRLLIYDASNRATGIPARFSGSGSGTDFTLTISSLEPEDFAVYYCQQRSNWPPTFGQGTKVEIKRTVAAPSVFIFPPSDEQLKSGTASVVCLLNNFYPREAKVQWKVDNALQSGNSQESVTEQDSKDSTYSLSSTLTLSKADYEKHKVYACEVTHQGLSSPVTKSFNRGEC

SEQ ID NO: 12 - protein, 471 aa, synthetic construct
MEFGLSWLFLVAILKGVQCEVQLLESGGGLVQPGGSLRLSCAVSGFTFNSFAMSWVRQAPGKGLEWVSAISGSGGGTYYADSVKGRFTISRDNSKNTLYLQMNSLRAEDTAVYFCAKDKILWFGEPVFDYWGQGTLVTVSSASTKGPSVFPLAPSSKSTSGGTAALGCLVKDYFPEPVTVSWNSGALTSGVHTFPAVLQSSGLYSLSSVVTVPSSSLGTQTYICNVNHKPSNTKVDKKVEPKSCDKTHTCPPCPAPELLGGPSVFLFPPKPKDTLMISRTPEVTCVVVDVSHEDPEVKFNWYVDGVEVHNAKTKPREEQYNSTYRVVSVLTVLHQDWLNGKEYKCKVSNKALPAPIEKTISKAKGQPREPQVYTLPPSREEMTKNQVSLSCAVKGFYPSDIAVEWESNGQPENNYKTTPPVLDSDGSFFLVSKLTVDKSRWQQGNVFSCSVMHEALHNRYTQKSLSLSPGK

SEQ ID NO: 13 - protein, 236 aa, synthetic construct
MDMRVPAQLLGLLLLWFPGSRCDIQMTQSPSSLSASVGDRVTITCKASQDVGIAVAWYQQKPGKVPKLLIYWASTRHTGVPDRFSGSGSGTDFTLTISSLQPEDVATYYCQQYSSYPYTFGQGTKVEIKRTVAAPSVFIFPPSDEQLKSGTASVVCLLNNFYPREAKVQWKVDNALQSGNSQESVTEQDSKDSTYSLSSTLTLSKADYEKHKVYACEVTHQGLSSPVTKSFNRGEC

SEQ ID NO: 14 - protein, 477 aa, synthetic construct
MEFGLSWLFLVAILKGVQCEVQLVESGGGLVQPGGSLRLSCAASGFDFSRYWMSWVRQAPGKGLEWIGEINPDSSTINYAPSLKDKFIISRDNAKNSLYLQMNSLRAEDTAVYYCARPDGNYWYFDVWGQGTLVTVSSASTKGPSVFPLAPSSKSTSGGTAALGCLVKDYFPEPVTVSWNSGALTSGVHTFPAVLQSSGLYSLSSVVTVPSSSLGTQTYICNVNHKPSNTKVDKKVEPKSCDKTHTCPPCPAPELLGGPSVFLFPPKPKDTLMISRTPEVTCVVVDVSHEDPEVKFNWYVDGVEVHNAKTKPREEQYNSTYRVVSVLTVLHQDWLNGKEYKCKVSNKALPAPIEKTISKAKGQPREPQVYTLPPSREEMTKNQVSLSCAVKGFYPSDIAVEWESNGQPENNYKTTPPVLDSDGSFFLVSKLTVDKSRWQQGNVFSCSVMHEALHNRYTQKSLSLSPGKGGSHHHHHH

SEQ ID NO: 15 - protein, 471 aa, synthetic construct
MEFGLSWLFLVAILKGVQCEVQLLESGGGLVQPGGSLRLSCAVSGFTFNSFAMSWVRQAPGKGLEWVSAISGSGGGTYYADSVKGRFTISRDNSKNTLYLQMNSLRAEDTAVYFCAKDKILWFGEPVFDYWGQGTLVTVSSASTKGPSVFPLAPSSKSTSGGTAALGCLVKDYFPEPVTVSWNSGALTSGVHTFPAVLQSSGLYSLSSVVTVPSSSLGTQTYICNVNHKPSNTKVDKKVEPKSCDKTHTCPPCPAPEAAGGPSVFLFPPKPKDTLMISRTPEVTCVVVDVSHEDPEVKFNWYVDGVEVHNAKTKPREEQYNSTYRVVSVLTVLHQDWLNGKEYKCKVSNKALPAPIEKTISKAKGQPREPQVYTLPPSREEMTKNQVSLSCAVKGFYPSDIAVEWESNGQPENNYKTTPPVLDSDGSFFLVSKLTVDKSRWQQGNVFSCSVMHEALHNRYTQKSLSLSPGK

SEQ ID NO: 16 - protein, 477 aa, synthetic construct
MEFGLSWLFLVAILKGVQCEVQLVESGGGLVQPGGSLRLSCAASGFDFSRYWMSWVRQAPGKGLEWIGEINPDSSTINYAPSLKDKFIISRDNAKNSLYLQMNSLRAEDTAVYYCARPDGNYWYFDVWGQGTLVTVSSASTKGPSVFPLAPSSKSTSGGTAALGCLVKDYFPEPVTVSWNSGALTSGVHTFPAVLQSSGLYSLSSVVTVPSSSLGTQTYICNVNHKPSNTKVDKKVEPKSCDKTHTCPPCPAPEAAGGPSVFLFPPKPKDTLMISRTPEVTCVVVDVSHEDPEVKFNWYVDGVEVHNAKTKPREEQYNSTYRVVSVLTVLHQDWLNGKEYKCKVSNKALPAPIEKTISKAKGQPREPQVYTLPPSREEMTKNQVSLSCAVKGFYPSDIAVEWESNGQPENNYKTTPPVLDSDGSFFLVSKLTVDKSRWQQGNVFSCSVMHEALHNRYTQKSLSLSPGKGGSHHHHHH

SEQ ID NO: 17 - protein, 242 aa, synthetic construct; identical to SEQ ID NO: 3

SEQ ID NO: 18 - protein, 471 aa, synthetic construct
MEFGLSWLFLVAILKGVQCQVQLVQSGAEVKKPGESVKVSCKASGYTFTNYGMNWVKQAPGQGLEWMGWINTYTGEPTYADKFQGRVTMTTDTSTSTAYMEIRNLGGDDTAVYYCARWSWSDGYYVYFDYWGQGTSVTVSSASTKGPSVFPLAPSSKSTSGGTAALGCLVKDYFPEPVTVSWNSGALTSGVHTFPAVLQSSGLYSLSSVVTVPSSSLGTQTYICNVNHKPSNTKVDKKVEPKSCDKTHTCPPCPAPELLGGPSVFLFPPKPKDTLMISRTPEVTCVVVDVSHEDPEVKFNWYVDGVEVHNAKTKPREEQYNSTYRVVSVLTVLHQDWLNGKEYKCKVSNKALPAPIEKTISKAKGQPREPQVYTLPPSRDELTKNQVSLTCLVKGFYPSDIAVEWESNGQPENNYKTTPPVLDSDGSFFLYSKLTVDKSRWQQGNVFSCSVMHEALHNHYTQKSLSLSPGK

SEQ ID NO: 19 - protein, 468 aa, synthetic construct
MEFGLSWLFLVAILKGVQCEVQLVESGGGLVQPGGSLRLSCAASGFDFSRYWMSWVRQAPGKGLEWIGEINPDSSTINYAPSLKDKFIISRDNAKNSLYLQMNSLRAEDTAVYYCARPDGNYWYFDVWGQGTLVTVSSASTKGPSVFPLAPSSKSTSGGTAALGCLVKDYFPEPVTVSWNSGALTSGVHTFPAVLQSSGLYSLSSVVTVPSSSLGTQTYICNVNHKPSNTKVDKKVEPKSCDKTHTCPPCPAPELLGGPSVFLFPPKPKDTLMISRTPEVTCVVVDVSHEDPEVKFNWYVDGVEVHNAKTKPREEQYNSTYRVVSVLTVLHQDWLNGKEYKCKVSNKALPAPIEKTISKAKGQPREPQVYTLPPSRDELTKNQVSLTCLVKGFYPSDIAVEWESNGQPENNYKTTPPVLDSDGSFFLYSKLTVDKSRWQQGNVFSCSVMHEALHNHYTQKSLSLSPGK

SEQ ID NO: 20 - protein, 236 aa, synthetic construct; identical to SEQ ID NO: 13

SEQ ID NO: 21 - protein, 471 aa, synthetic construct
MEFGLSWLFLVAILKGVQCEVQLLESGGGLVQPGGSLRLSCAVSGFTFNSFAMSWVRQAPGKGLEWVSAISGSGGGTYYADSVKGRFTISRDNSKNTLYLQMNSLRAEDTAVYFCAKDKILWFGEPVFDYWGQGTLVTVSSASTKGPSVFPLAPSSKSTSGGTAALGCLVKDYFPEPVTVSWNSGALTSGVHTFPAVLQSSGLYSLSSVVTVPSSSLGTQTYICNVNHKPSNTKVDKKVEPKSCDKTHTCPPCPAPELLGGPSVFLFPPKPKDTLMISRTPEVTCVVVDVSHEDPEVKFNWYVDGVEVHNAKTKPREEQYNSTYRVVSVLTVLHQDWLNGKEYKCKVSNKALPAPIEKTISKAKGQPREPQVYTLPPSRDELTKNQVSLTCLVKGFYPSDIAVEWESNGQPENNYKTTPPVLDSDGSFFLYSKLTVDKSRWQQGNVFSCSVMHEALHNHYTQKSLSLSPGK

SEQ ID NO: 22 - protein, 236 aa, synthetic construct; identical to SEQ ID NO: 11

SEQ ID NO: 23 - protein, 469 aa, synthetic construct
MEFGLSWLFLVAILKGVQCQVQLVQSGAEVKKPGESLKVSCKASGYTFTSYYMHWVRQAPGQGLEWMGIINPSGGSTSYAQKFQGRVTMTRDTSTSTVYMELSSLRSEDTAVYYCARGSAYYYDFADYWGQGTLVTVSSASTKGPSVFPLAPSSKSTSGGTAALGCLVKDYFPEPVTVSWNSGALTSGVHTFPAVLQSSGLYSLSSVVTVPSSSLGTQTYICNVNHKPSNTKVDKKVEPKSCDKTHTCPPCPAPEAAGGPSVFLFPPKPKDTLMISRTPEVTCVVVDVSHEDPEVKFNWYVDGVEVHNAKTKPREEQYNSTYRVVSVLTVLHQDWLNGKEYKCKVSNKALPAPIEKTISKAKGQPREPQVYTLPPSRDELTKNQVSLTCLVKGFYPSDIAVEWESNGQPENNYKTTPPVLDSDGSFFLYSKLTVDKSRWQQGNVFSCSVMHEALHNHYTQKSLSLSPGK

SEQ ID NO: 24 - protein, 235 aa, synthetic construct
MDMRVPAQLLGLLLLWFPGSRCSYVLTQPSSVSVAPGQTATISCGGHNIGSKNVHWYQQRPGQSPVLVIYQDNKRPSGIPERFSGSNSGNTATLTISGTQAMDEADYYCQVWDNYSVLFGGGTKLTVLRTVAAPSVFIFPPSDEQLKSGTASVVCLLNNFYPREAKVQWKVDNALQSGNSQESVTEQDSKDSTYSLSSTLTLSKADYEKHKVYACEVTHQGLSSPVTKSFNRGEC

SEQ ID NO: 25 - protein, 508 aa, synthetic construct
MEFGLSWLFLVAILKGVQCQVQLVQSGAEVKKPGESLKVSCKASGYTFTSYYMHWVRQAPGQGLEWMGIINPSGGSTSYAQKFQGRVTMTRDTSTSTVYMELSSLRSEDTAVYYCARGSAYYYDFADYWGQGTLVTVSSGGGGSGGGGSGGGGSSYVLTQPSSVSVAPGQTATISCGGHNIGSKNVHWYQQRPGQSPVLVIYQDNKRPSGIPERFSGSNSGNTATLTISGTQAMDEADYYCQVWDNYSVLFGGGTKLTVLGGGGSEPKSSDKTHTCPPCPAPELLGGPSVFLFPPKPKDTLMISRTPEVTCVVVDVSHEDPEVKFNWYVDGVEVHNAKTKPREEQYNSTYRVVSVLTVLHQDWLNGKEYKCKVSNKALPAPIEKTISKAKGQPREPQVYTLPPSRDELTKNQVSLWCLVKGFYPSDIAVEWESNGQPENNYKTTPPVLDSDGSFFLYSKLTVDKSRWQQGNVFSCSVMHEALHNHYTQKSLSLSPGKGGSDYKDDDDK

SEQ ID NO: 26 - protein, 480 aa, synthetic construct
MEFGLSWLFLVAILKGVQCQVQLVQSGAEVKKPGESVKVSCKASGYTFTNYGMNWVKQAPGQGLEWMGWINTYTGEPTYADKFQGRVTMTTDTSTSTAYMEIRNLGGDDTAVYYCARWSWSDGYYVYFDYWGQGTSVTVSSASTKGPSVFPLAPSSKSTSGGTAALGCLVKDYFPEPVTVSWNSGALTSGVHTFPAVLQSSGLYSLSSVVTVPSSSLGTQTYICNVNHKPSNTKVDKKVEPKSCDKTHTCPPCPAPELLGGPSVFLFPPKPKDTLMISRTPEVTCVVVDVSHEDPEVKFNWYVDGVEVHNAKTKPREEQYNSTYRVVSVLTVLHQDWLNGKEYKCKVSNKALPAPIEKTISKAKGQPREPQVYTLPPSREEMTKNQVSLSCAVKGFYPSDIAVEWESNGQPENNYKTTPPVLDSDGSFFLVSKLTVDKSRWQQGNVFSCSVMHEALHNRYTQKSLSLSPGKGGSHHHHHH

SEQ ID NO: 27 - protein, 242 aa, synthetic construct; identical to SEQ ID NO: 3

SEQ ID NO: 28 - protein, 508 aa, synthetic construct; identical to SEQ ID NO: 25

SEQ ID NO: 29 - protein, 480 aa, synthetic construct; identical to SEQ ID NO: 26

SEQ ID NO: 30 - protein, 242 aa, synthetic construct; identical to SEQ ID NO: 3

SEQ ID NO: 31 - protein, 641 aa, synthetic construct
MEFGLSWLFLVAILKGVQCEVQLVESGGGVVRPGGSLRLSCAASGFTFDDYGMSWVRQAPGKGLEWVSGINWNGGSTGYADSVKGRFTISRDNAKNSLYLQMNSLRAEDTAVYYCARGRSLLFDYWGQGTLVTVSRGGGGSGGGGSGGGGSSELTQDPAVSVALGQTVRITCQGDSLRSYYASWYQQKPGQAPVLVIYGKNNRPSGIPDRFSGSSSGNTASLTITGAQAEDEADYYCNSRDSSGNHVVFGGGTKLTVLPSGQAGAAASESLFVSNHAYNWVNVISDLKKIEDLIQSMHIDATLYTESDVHPSCKVTAMKCFLLELQVISLESGDASIHDTVENLIILANDSLSSNGNVTESGCKECEELEEKNIKEFLQSFVHIVQMFINTSEASGGPEQVQLVQSGAEVKKPGSSVKVSCKASGYTFTDYNMHWVRQAPGQGLEWIGYIYPYNGGTGYNQKFKSKATITADESTNTAYMELSSLRSEDTAVYYCARGRPAMDYWGQGTLVTVSSGGGGSGGGGSGGGGSDIQMTQSPSSLSASVGDRVTITCRASESVDNYGISFMNWFQQKPGKAPKLLIYAASNQGSGVPSRFSGSGSGTDFTLTISSLQPDDFATYYCQQSKEVPWTFGQGTKVEIK

SEQ ID NO: 32 - protein, 133 aa, synthetic construct
MEFGLSWLFLVAILKGVQCNWVNVISDLKKIEDLIQSMHIDATLYTESDVHPSCKVTAMKCFLLELQVISCESGDASIHDTVENLIILANNSLSSNGNVTESGCKECEELEEKNIKEFLQSFVHIVQMFINTS

SEQ ID NO: 33 - protein, 344 aa, synthetic construct
MEFGLSWLFLVAILKGVQCITCPPPMSVEHADIWVKSYSLYSRERYICNSGFKRKAGTCSLTECVLNKATNVAHWTTPSLKCIRDPALVHQRSGGSGGGGSGGGSGGGGSLQEPKSSDKTHTCPPCPAPELLGGPSVFLFPPKPKDTLMISRTPEVTCVVVDVSHEDPEVKFNWYVDGVEVHNAKTKPREEQYNSTYRVVSVLTVLHQDWLNGKEYKCKVSNKALPAPIEKTISKAKGQPREPQVYTLPPSRDELTKNQVSLTCLVKGFYPSDIAVEWESNGQPENNYKTTPPVLDSDGSFFLYSKLTVDKSRWQQGNVFSCSVMHEALHNHYTQKSLSLSPGK

SEQ ID NO: 34 - protein, 508 aa, synthetic construct; identical to SEQ ID NO: 25

SEQ ID NO: 35 - protein, 477 aa, synthetic construct; identical to SEQ ID NO: 16

SEQ ID NO: 36 - protein, 508 aa, synthetic construct; identical to SEQ ID NO: 25

SEQ ID NO: 37 - protein, 480 aa, synthetic construct
MEFGLSWLFLVAILKGVQCEVQLLESGGGLVQPGGSLRLSCAVSGFTFNSFAMSWVRQAPGKGLEWVSAISGSGGGTYYADSVKGRFTISRDNSKNTLYLQMNSLRAEDTAVYFCAKDKILWFGEPVFDYWGQGTLVTVSSASTKGPSVFPLAPSSKSTSGGTAALGCLVKDYFPEPVTVSWNSGALTSGVHTFPAVLQSSGLYSLSSVVTVPSSSLGTQTYICNVNHKPSNTKVDKKVEPKSCDKTHTCPPCPAPEAAGGPSVFLFPPKPKDTLMISRTPEVTCVVVDVSHEDPEVKFNWYVDGVEVHNAKTKPREEQYNSTYRVVSVLTVLHQDWLNGKEYKCKVSNKALPAPIEKTISKAKGQPREPQVYTLPPSREEMTKNQVSLSCAVKGFYPSDIAVEWESNGQPENNYKTTPPVLDSDGSFFLVSKLTVDKSRWQQGNVFSCSVMHEALHNRYTQKSLSLSPGKGGSHHHHHH

SEQ ID NO: 38 - protein, 220 aa, synthetic construct
DIVMTQSPDSLTVSLGERTTINCKSSQSVLDSSTNKNSLAWYQQKPGQPPKLLLSWASTRESGIPDRFSGSGSGTDFTLTIDSPQPEDSATYYCQQSAHFPITFGQGTRLEIKRTVAAPSVFIFPPSDEQLKSGTASVVCLLNNFYPREAKVQWKVDNALQSGNSQESVTEQDSKDSTYSLSSTLTLSKADYEKHKVYACEVTHQGLSSPVTKSFNRGEC

SEQ ID NO: 39 - protein, 461 aa, synthetic construct
QVQLVQSGAEVKKPGESVKVSCKASGYTFTNYGMNWVKQAPGQGLEWMGWINTYTGEPTYADKFQGRVTMTTDTSTSTAYMEIRNLGGDDTAVYYCARWSWSDGYYVYFDYWGQGTSVTVSSASTKGPSVFPLAPSSKSTSGGTAALGCLVKDYFPEPVTVSWNSGALTSGVHTFPAVLQSSGLYSLSSVVTVPSSSLGTQTYICNVNHKPSNTKVDKKVEPKSCDKTHTCPPCPAPEAAGGPSVFLFPPKPKDTLMISRTPEVTCVVVDVSHEDPEVKFNWYVDGVEVHNAKTKPREEQYNSTYRVVSVLTVLHQDWLNGKEYKCKVSNKALPAPIEKTISKAKGQPREPQVYTLPPSREEMTKNQVSLSCAVKGFYPSDIAVEWESNGQPENNYKTTPPVLDSDGSFFLVSKLTVDKSRWQQGNVFSCSVMHEALHNRYTQKSLSLSPGKGGSHHHHHH

SEQ ID NO: 40 - protein, 572 aa, synthetic construct
MEFGLSWLFLVAILKGVQCQVQLVQSGAEVKKPGESVKVSCKASGYTFTNYGMNWVKQAPGQGLEWMGWINTYTGEPTYADKFQGRVTMTTDTSTSTAYMEIRNLGGDDTAVYYCARWSWSDGYYVYFDYWGQGTSVTVSSGGGSGGGGSYVLTQPSSVSVAPGQTATISCGGHNIGSKNVHWYQQRPGQSPVLVIYQDNKRPSGIPERFSGSNSGNTATLTISGTQAMDEADYYCQVWDNYSVLFGGGTKLTVLGGGGSGGGGSGGGGSITCPPPMSVEHADIWVKSYSLYSRERYICNSGFKRKAGTCSLTECVLNKATNVAHWTTPSLKCIRGGGGSEPKSSDKTHTCPPCPAPEAAGGPSVFLFPPKPKDTLMISRTPEVTCVVVDVSHEDPEVKFNWYVDGVEVHNAKTKPREEQYNSTYRVVSVLTVLHQDWLNGKEYKCKVSNKALPAPIEKTISKAKGQPREPQVYTLPPSRDELTKNQVSLWCLVKGFYPSDIAVEWESNGQPENNYKTTPPVLDSDGSFFLYSKLTVDKSRWQQGNVFSCSVMHEALHNHYTQKSLSLSPGK

SEQ ID NO: 41 - protein, 389 aa, synthetic construct
MEFGLSWLFLVAILKGVQCQVQLVQSGAEVKKPGESLKVSCKASGYTFTSYYMHWVRQAPGQGLEWMGIINPSGGSTSYAQKFQGRVTMTRDTSTSTVYMELSSLRSEDTAVYYCARGSAYYYDFADYWGQGTLVTVSSGGGSGGGGDIVMTQSPDSLTVSLGERTTINCKSSQSVLDSSTNKNSLAWYQQKPGQPPKLLLSWASTRESGIPDRFSGSGSGTDFTLTIDSPQPEDSATYYCQQSAHFPITFGQGTRLEIKGGGGSGGGGSGGGGSNWVNVISDLKKIEDLIQSMHIDATLYTESDVHPSCKVTAMKCFLLELQVISCESGDASIHDTVENLIILANNSLSSNGNVTESGCKECEELEEKNIKEFLQSFVHIVQMFINTS

SEQ ID NO: 42 - protein, 588 aa, synthetic construct
MEFGLSWLFLVAILKGVQCQVQLVQSGAEVKKPGESLKVSCKASGYTFTSYYMHWVRQAPGQGLEWMGIINPSGGSTSYAQKFQGRVTMTRDTSTSTVYMELSSLRSEDTAVYYCARGSAYYYDFADYWGQGTLVTVSSGGGSGGGGDIVMTQSPDSLTVSLGERTTINCKSSQSVLDSSTNKNSLAWYQQKPGQPPKLLLSWASTRESGIPDRFSGSGSGTDFTLTIDSPQPEDSATYYCQQSAHFPITFGQGTRLEIKGGGGSGGGGSGGGGSITCPPPMSVEHADIWVKSYSLYSRERYICNSGFKRKAGTCSLTECVLNKATNVAHWTTPSLKCIRGGGGSEPKSSDKTHTCPPCPAPEAAGGPSVFLFPPKPKDTLMISRTPEVTCVVVDVSHEDPEVKFNWYVDGVEVHNAKTKPREEQYNSTYRVVSVLTVLHQDWLNGKEYKCKVSNKALPAPIEKTISKAKGQPREPQVYTLPPSRDELTKNQVSLWCLVKGFYPSDIAVEWESNGQPENNYKTTPPVLDSDGSFFLYSKLTVDKSRWQQGNVFSCSVMHEALHNHYTQKSLSLSPGKGGSDYKDDDDK

SEQ ID NO: 43 - protein, 384 aa, synthetic construct
MEFGLSWLFLVAILKGVQCQVQLVQSGAEVKKPGESVKVSCKASGYTFTNYGMNWVKQAPGQGLEWMGWINTYTGEPTYADKFQGRVTMTTDTSTSTAYMEIRNLGGDDTAVYYCARWSWSDGYYVYFDYWGQGTSVTVSSGGGSGGGGSYVLTQPSSVSVAPGQTATISCGGHNIGSKNVHWYQQRPGQSPVLVIYQDNKRPSGIPERFSGSNSGNTATLTISGTQAMDEADYYCQVWDNYSVLFGGGTKLTVLGGGGSGGGGSGGGGSNWVNVISDLKKIEDLIQSMHIDATLYTESDVHPSCKVTAMKCFLLELQVISCESGDASIHDTVENLIILANNSLSSNGNVTESGCKECEELEEKNIKEFLQSFVHIVQMFINTS

SEQ ID NO: 44 - protein, 392 aa, synthetic construct
MDMRVPAQLLGLLLLWFPGSRCDIVMTQSPDSLTVSLGERTTINCKSSQSVLDSSTNKNSLAWYQQKPGQPPKLLLSWASTRESGIPDRFSGSGSGTDFTLTIDSPQPEDSATYYCQQSAHFPITFGQGTRLEIKGGGSGGGGQVQLVQSGAEVKKPGESLKVSCKASGYTFTSYYMHWVRQAPGQGLEWMGIINPSGGSTSYAQKFQGRVTMTRDTSTSTVYMELSSLRSEDTAVYYCARGSAYYYDFADYWGQGTLVTVSSGGGGSGGGGSGGGGSNWVNVISDLKKIEDLIQSMHIDATLYTESDVHPSCKVTAMKCFLLELQVISCESGDASIHDTVENLIILANNSLSSNGNVTESGCKECEELEEKNIKEFLQSFVHIVQMFINTS

SEQ ID NO: 45 - protein, 575 aa, synthetic construct
MDMRVPAQLLGLLLLWFPGSRCSYVLTQPSSVSVAPGQTATISCGGHNIGSKNVHWYQQRPGQSPVLVIYQDNKRPSGIPERFSGSNSGNTATLTISGTQAMDEADYYCQVWDNYSVLFGGGTKLTVLGGGSGGGGQVQLVQSGAEVKKPGESVKVSCKASGYTFTNYGMNWVKQAPGQGLEWMGWINTYTGEPTYADKFQGRVTMTTDTSTSTAYMEIRNLGGDDTAVYYCARWSWSDGYYVYFDYWGQGTSVTVSSGGGGSGGGGSGGGGSITCPPPMSVEHADIWVKSYSLYSRERYICNSGFKRKAGTCSLTECVLNKATNVAHWTTPSLKCIRGGGGSEPKSSDKTHTCPPCPAPEAAGGPSVFLFPPKPKDTLMISRTPEVTCVVVDVSHEDPEVKFNWYVDGVEVHNAKTKPREEQYNSTYRVVSVLTVLHQDWLNGKEYKCKVSNKALPAPIEKTISKAKGQPREPQVYTLPPSRDELTKNQVSLWCLVKGFYPSDIAVEWESNGQPENNYKTTPPVLDSDGSFFLYSKLTVDKSRWQQGNVFSCSVMHEALHNHYTQKSLSLSPGK

SEQ ID NO: 46 - protein, 590 aa, synthetic construct
MDMRVPAQLLGLLLLWFPGSRCDIVMTQSPDSLTVSLGERTTINCKSSQSVLDSSTNKNSLAWYQQKPGQPPKLLLSWASTRESGIPDRFSGSGSGTDFTLTIDSPQPEDSATYYCQQSAHFPITFGQGTRLEIKGGGSGGGGQVQLVQSGAEVKKPGESLKVSCKASGYTFTSYYMHWVRQAPGQGLEWMGIINPSGGSTSYAQKFQGRVTMTRDTSTSTVYMELSSLRSEDTAVYYCARGSAYYYDFADYWGQGTLVTVSSGGGGSGGGGSGGGGSITCPPPMSVEHADIWVKSYSLYSRERYICNSGFKRKAGTCSLTECVLNKATNVAHWTTPSLKCIRGGGGSEPKSSDKTHTCPPCPAPEAAGGPSVFLFPPKPKDTLMISRTPEVTCVVVDVSHEDPEVKFNWYVDGVEVHNAKTKPREEQYNSTYRVVSVLTVLHQDWLNGKEYKCKVSNKALPAPIEKTISKAKGQPREPQVYTLPPSRDELTKNQVSLWCLVKGFYPSDIAVEWESNGQPENNYKTTPPVLDSDGSFFLYSKLTVDKSRWQQGNVFSCSVMHEALHNHYTQKSLSLSPGKGGSDYKDDDK

SEQ ID NO: 47 - protein, 387 aa, synthetic construct
MDMRVPAQLLGLLLLWFPGSRCSYVLTQPSSVSVAPGQTATISCGGHNIGSKNVHWYQQRPGQSPVLVIYQDNKRPSGIPERFSGSNSGNTATLTISGTQAMDEADYYCQVWDNYSVLFGGGTKLTVLGGGSGGGGQVQLVQSGAEVKKPGESVKVSCKASGYTFTNYGMNWVKQAPGQGLEWMGWINTYTGEPTYADKFQGRVTMTTDTSTSTAYMEIRNLGGDDTAVYYCARWSWSDGYYVYFDYWGQGTSVTVSSGGGGSGGGGSGGGGSNWVNVISDLKKIEDLIQSMHIDATLYTESDVHPSCKVTAMKCFLLELQVISCESGDASIHDTVENLIILANNSLSSNGNVTESGCKECEELEEKNIKEFLQSFVHIVQMFINTS

SEQ ID NO: 48 - protein, 214 aa, synthetic construct
EIVLTQSPATLSLSPGERATLSCRASQSVSSYLAWYQQKPGQAPRLLIYDASNRATGIPARFSGSGSGTDFTLTISSLEPEDFAVYYCQQRSNWPPTFGQGTKVEIKRTVAAPSVFIFPPSDEQLKSGTASVVCLLNNFYPREAKVQWKVDNALQSGNSQESVTEQDSKDSTYSLSSTLTLSKADYEKHKVYACEVTHQGLSSPVTKSFNRGEC

SEQ ID NO: 49 - protein, 461 aa, synthetic construct
EVQLLESGGGLVQPGGSLRLSCAVSGFTFNSFAMSWVRQAPGKGLEWVSAISGSGGGTYYADSVKGRFTISRDNSKNTLYLQMNSLRAEDTAVYFCAKDKILWFGEPVFDYWGQGTLVTVSSASTKGPSVFPLAPSSKSTSGGTAALGCLVKDYFPEPVTVSWNSGALTSGVHTFPAVLQSSGLYSLSSVVTVPSSSLGTQTYICNVNHKPSNTKVDKKVEPKSCDKTHTCPPCPAPEAAGGPSVFLFPPKPKDTLMISRTPEVTCVVVDVSHEDPEVKFNWYVDGVEVHNAKTKPREEQYNSTYRVVSVLTVLHQDWLNGKEYKCKVSNKALPAPIEKTISKAKGQPREPQVYTLPPSREEMTKNQVSLSCAVKGFYPSDIAVEWESNGQPENNYKTTPPVLDSDGSFFLVSKLTVDKSRWQQGNVFSCSVMHEALHNRYTQKSLSLSPGKGGSHHHHHH

SEQ ID NO: 50 - protein, 580 aa, synthetic construct
MEFGLSWLFLVAILKGVQCEVQLVESGGGLVQPGGSLRLSCAASGFDFSRYWMSWVRQAPGKGLEWIGEINPDSSTINYAPSLKDKFIISRDNAKNSLYLQMNSLRAEDTAVYYCARPDGNYWYFDVWGQGTLVTVSSGGGSGGGGSYVLTQPSSVSVAPGQTATISCGGHNIGSKNVHWYQQRPGQSPVLVIYQDNKRPSGIPERFSGSNSGNTATLTISGTQAMDEADYYCQVWDNYSVLFGGGTKLTVLGGGGSGGGGSGGGGSITCPPPMSVEHADIWVKSYSLYSRERYICNSGFKRKAGTCSLTECVLNKATNVAHWTTPSLKCIRGGGGSEPKSSDKTHTCPPCPAPEAAGGPSVFLFPPKPKDTLMISRTPEVTCVVVDVSHEDPEVKFNWYVDGVEVHNAKTKPREEQYNSTYRVVSVLTVLHQDWLNGKEYKCKVSNKALPAPIEKTISKAKGQPREPQVYTLPPSRDELTKNQVSLWCLVKGFYPSDIAVEWESNGQPENNYKTTPPVLDSDGSFFLYSKLTVDKSRWQQGNVFSCSVMHEALHNHYTQKSLSLSPGKGGSDYKDDDDK

SEQ ID NO: 51 - protein, 383 aa, synthetic construct
MEFGLSWLFLVAILKGVQCQVQLVQSGAEVKKPGESLKVSCKASGYTFTSYYMHWVRQAPGQGLEWMGIINPSGGSTSYAQKFQGRVTMTRDTSTSTVYMELSSLRSEDTAVYYCARGSAYYYDFADYWGQGTLVTVSSGGGSGGGGDIQMTQSPSSLSASVGDRVTITCKASQDVGIAVAWYQQKPGKVPKLLIYWASTRHTGVPDRFSGSGSGTDFTLTISSLQPEDVATYYCQQYSSYPYTFGQGTKVEIKGGGGSGGGGSGGGGSNWVNVISDLKKIEDLIQSMHIDATLYTESDVHPSCKVTAMKCFLLELQVISCESGDASIHDTVENLIILANNSLSSNGNVTESGCKECEELEEKNIKEFLQSFVHIVQMFINTS

SEQ ID NO: 52 - protein, 571 aa, synthetic construct
MEFGLSWLFLVAILKGVQCQVQLVQSGAEVKKPGESLKVSCKASGYTFTSYYMHWVRQAPGQGLEWMGIINPSGGSTSYAQKFQGRVTMTRDTSTSTVYMELSSLRSEDTAVYYCARGSAYYYDFADYWGQGTLVTVSSGGGSGGGGDIQMTQSPSSLSASVGDRVTITCKASQDVGIAVAWYQQKPGKVPKLLIYWASTRHTGVPDRFSGSGSGTDFTLTISSLQPEDVATYYCQQYSSYPYTFGQGTKVEIKGGGGSGGGGSGGGGSITCPPPMSVEHADIWVKSYSLYSRERYICNSGFKRKAGTCSLTECVLNKATNVAHWTTPSLKCIRGGGGSEPKSSDKTHTCPPCPAPEAAGGPSVFLFPPKPKDTLMISRTPEVTCVVVDVSHEDPEVKFNWYVDGVEVHNAKTKPREEQYNSTYRVVSVLTVLHQDWLNGKEYKCKVSNKALPAPIEKTISKAKGQPREPQVYTLPPSRDELTKNQVSLWCLVKGFYPSDIAVEWESNGQPENNYKTTPPVLDSDGSFFLYSKLTVDKSRWQQGNVFSCSVMHEALHNHYTQKSLSLSPGK

SEQ ID NO: 53 - protein, 381 aa, synthetic construct
MEFGLSWLFLVAILKGVQCEVQLVESGGGLVQPGGSLRLSCAASGFDFSRYWMSWVRQAPGKGLEWIGEINPDSSTINYAPSLKDKFIISRDNAKNSLYLQMNSLRAEDTAVYYCARPDGNYWYFDVWGQGTLVTVSSGGGSGGGGSYVLTQPSSVSVAPGQTATISCGGHNIGSKNVHWYQQRPGQSPVLVIYQDNKRPSGIPERFSGSNSGNTATLTISGTQAMDEADYYCQVWDNYSVLFGGGTKLTVLGGGGSGGGGSGGGGSNWVNVISDLKKIEDLIQSMHIDATLYTESDVHPSCKVTAMKCFLLELQVISCESGDASIHDTVENLIILANNSLSSNGNVTESGCKECEELEEKNIKEFLQSFVHIVQMFINTS

SEQ ID NO: 54 - protein, 583 aa, synthetic construct
MDMRVPAQLLGLLLLWFPGSRCSYVLTQPSSVSVAPGQTATISCGGHNIGSKNVHWYQQRPGQSPVLVIYQDNKRPSGIPERFSGSNSGNTATLTISGTQAMDEADYYCQVWDNYSVLFGGGTKLTVLGGGSGGGGEVQLVESGGGLVQPGGSLRLSCAASGFDFSRYWMSWVRQAPGKGLEWIGEINPDSSTINYAPSLKDKFIISRDNAKNSLYLQMNSLRAEDTAVYYCARPDGNYWYFDVWGQGTLVTVSSGGGGSGGGGSGGGGSITCPPPMSVEHADIWVKSYSLYSRERYICNSGFKRKAGTCSLTECVLNKATNVAHWTTPSLKCIRGGGGSEPKSSDKTHTCPPCPAPEAAGGPSVFLFPPKPKDTLMISRTPEVTCVVVDVSHEDPEVKFNWYVDGVEVHNAKTKPREEQYNSTYRVVSVLTVLHQDWLNGKEYKCKVSNKALPAPIEKTISKAKGQPREPQVYTLPPSRDELTKNQVSLWCLVKGFYPSDIAVEWESNGQPENNYKTTPPVLDSDGSFFLYSKLTVDKSRWQQGNVFSCSVMHEALHNHYTQKSLSLSPGKGGSDYKDDDDK

SEQ ID NO: 55 - protein, 386 aa, synthetic construct
MDMRVPAQLLGLLLLWFPGSRCDIQMTQSPSSLSASVGDRVTITCKASQDVGIAVAWYQQKPGKVPKLLIYWASTRHTGVPDRFSGSGSGTDFTLTISSLQPEDVATYYCQQYSSYPYTFGQGTKVEIKGGGSGGGGQVQLVQSGAEVKKPGESLKVSCKASGYTFTSYYMHWVRQAPGQGLEWMGIINPSGGSTSYAQKFQGRVTMTRDTSTSTVYMELSSLRSEDTAVYYCARGSAYYYDFADYWGQGTLVTVSSGGGGSGGGGSGGGGSNWVNVISDLKKIEDLIQSMHIDATLYTESDVHPSCKVTAMKCFLLELQVISCESGDASIHDTVENLIILANNSLSSNGNVTESGCKECEELEEKNIKEFLQSFVHIVQMFINTS

SEQ ID NO: 56 - protein, 585 aa, synthetic construct
MDMRVPAQLLGLLLLWFPGSRCDIQMTQSPSSLSASVGDRVTITCKASQDVGIAVAWYQQKPGKVPKLLIYWASTRHTGVPDRFSGSGSGTDFTLTISSLQPEDVATYYCQQYSSYPYTFGQGTKVEIKGGGSGGGGQVQLVQSGAEVKKPGESLKVSCKASGYTFTSYYMHWVRQAPGQGLEWMGIINPSGGSTSYAQKFQGRVTMTRDTSTSTVYMELSSLRSEDTAVYYCARGSAYYYDFADYWGQGTLVTVSSGGGGSGGGGSGGGGSITCPPPMSVEHADIWVKSYSLYSRERYICNSGFKRKAGTCSLTECVLNKATNVAHWTTPSLKCIRGGGGSEPKSSDKTHTCPPCPAPEAAGGPSVFLFPPKPKDTLMISRTPEVTCVVVDVSHEDPEVKFNWYVDGVEVHNAKTKPREEQYNSTYRVVSVLTVLHQDWLNGKEYKCKVSNKALPAPIEKTISKAKGQPREPQVYTLPPSRDELTKNQVSLWCLVKGFYPSDIAVEWESNGQPENNYKTTPPVLDSDGSFFLYSKLTVDKSRWQQGNVFSCSVMHEALHNHYTQKSLSLSPGKGGSDYKDDDDK

SEQ ID NO: 57 - protein, 384 aa, synthetic construct
MDMRVPAQLLGLLLLWFPGSRCSYVLTQPSSVSVAPGQTATISCGGHNIGSKNVHWYQQRPGQSPVLVIYQDNKRPSGIPERFSGSNSGNTATLTISGTQAMDEADYYCQVWDNYSVLFGGGTKLTVLGGGSGGGGEVQLVESGGGLVQPGGSLRLSCAASGFDFSRYWMSWVRQAPGKGLEWIGEINPDSSTINYAPSLKDKFIISRDNAKNSLYLQMNSLRAEDTAVYYCARPDGNYWYFDVWGQGTLVTVSSGGGGSGGGGSGGGGSNWVNVISDLKKIEDLIQSMHIDATLYTESDVHPSCKVTAMKCFLLELQVISCESGDASIHDTVENLIILANNSLSSNGNVTESGCKECEELEEKNIKEFLQSFVHIVQMFINTS

SEQ ID NO: 58 - protein, 214 aa, synthetic construct
DIQMTQSPSSLSASVGDRVTITCKASQDVGIAVAWYQQKPGKVPKLLIYWASTRHTGVPDRFSGSGSGTDFTLTISSLQPEDVATYYCQQYSSYPYTFGQGTKVEIKRTVAAPSVFIFPPSDEQLKSGTASVVCLLNNFYPREAKVQWKVDNALQSGNSQESVTEQDSKDSTYSLSSTLTLSKADYEKHKVYACEVTHQGLSSPVTKSFNRGEC

SEQ ID NO: 59 - protein, 449 aa, synthetic construct
EVQLVESGGGLVQPGGSLRLSCAASGFDFSRYWMSWVRQAPGKGLEWIGEINPDSSTINYAPSLKDKFIISRDNAKNSLYLQMNSLRAEDTAVYYCARPDGNYWYFDVWGQGTLVTVSSASTKGPSVFPLAPSSKSTSGGTAALGCLVKDYFPEPVTVSWNSGALTSGVHTFPAVLQSSGLYSLSSVVTVPSSSLGTQTYICNVNHKPSNTKVDKKVEPKSCDKTHTCPPCPAPEAAGGPSVFLFPPKPKDTLMISRTPEVTCVVVDVSHEDPEVKFNWYVDGVEVHNAKTKPREEQYNSTYRVVSVLTVLHQDWLNGKEYKCKVSNKALPAPIEKTISKAKGQPREPQVYTLPPSREEMTKNQVSLSCAVKGFYPSDIAVEWESNGQPENNYKTTPPVLDSDGSFFLVSKLTVDKSRWQQGNVFSCSVMHEALHNRYTQKSLSLSPGK

SEQ ID NO: 60 - protein, 583 aa, synthetic construct
MEFGLSWLFLVAILKGVQCEVQLLESGGGLVQPGGSLRLSCAVSGFTFNSFAMSWVRQAPGKGLEWVSAISGSGGGTYYADSVKGRFTISRDNSKNTLYLQMNSLRAEDTAVYFCAKDKILWFGEPVFDYWGQGTLVTVSSGGGSGGGGSYVLTQPSSVSVAPGQTATISCGGHNIGSKNVHWYQQRPGQSPVLVIYQDNKRPSGIPERFSGSNSGNTATLTISGTQAMDEADYYCQVWDNYSVLFGGGTKLTVLGGGGSGGGGSGGGGSITCPPPMSVEHADIWVKSYSLYSRERYICNSGFKRKAGTCSLTECVLNKATNVAHWTTPSLKCIRGGGGSEPKSSDKTHTCPPCPAPEAAGGPSVFLFPPKPKDTLMISRTPEVTCVVVDVSHEDPEVKFNWYVDGVEVHNAKTKPREEQYNSTYRVVSVLTVLHQDWLNGKEYKCKVSNKALPAPIEKTISKAKGQPREPQVYTLPPSRDELTKNQVSLWCLVKGFYPSDIAVEWESNGQPENNYKTTPPVLDSDGSFFLYSKLTVDKSRWQQGNVFSCSVMHEALHNHYTQKSLSLSPGKGGSDYKDDDDK

SEQ ID NO: 61 - protein, 383 aa, synthetic construct
MEFGLSWLFLVAILKGVQCQVQLVQSGAEVKKPGESLKVSCKASGYTFTSYYMHWVRQAPGQGLEWMGIINPSGGSTSYAQKFQGRVTMTRDTSTSTVYMELSSLRSEDTAVYYCARGSAYYYDFADYWGQGTLVTVSSGGGSGGGGEIVLTQSPATLSLSPGERATLSCRASQSVSSYLAWYQQKPGQAPRLLIYDASNRATGIPARFSGSGSGTDFTLTISSLEPEDFAVYYCQQRSNWPPTFGQGTKVEIKGGGGSGGGGSGGGGSNWVNVISDLKKIEDLIQSMHIDATLYTESDVHPSCKVTAMKCFLLELQVISCESGDASIHDTVENLIILANNSLSSNGNVTESGCKECEELEEKNIKEFLQSFVHIVQMFINTS

SEQ ID NO: 62 - protein, 582 aa, synthetic construct
MEFGLSWLFLVAILKGVQCQVQLVQSGAEVKKPGESLKVSCKASGYTFTSYYMHWVRQAPGQGLEWMGIINPSGGSTSYAQKFQGRVTMTRDTSTSTVYMELSSLRSEDTAVYYCARGSAYYYDFADYWGQGTLVTVSSGGGSGGGGEIVLTQSPATLSLSPGERATLSCRASQSVSSYLAWYQQKPGQAPRLLIYDASNRATGIPARFSGSGSGTDFTLTISSLEPEDFAVYYCQQRSNWPPTFGQGTKVEIKGGGGSGGGGSGGGGSITCPPPMSVEHADIWVKSYSLYSRERYICNSGFKRKAGTCSLTECVLNKATNVAHWTTPSLKCIRGGGGSEPKSSDKTHTCPPCPAPEAAGGPSVFLFPPKPKDTLMISRTPEVTCVVVDVSHEDPEVKFNWYVDGVEVHNAKTKPREEQYNSTYRVVSVLTVLHQDWLNGKEYKCKVSNKALPAPIEKTISKAKGQPREPQVYTLPPSRDELTKNQVSLWCLVKGFYPSDIAVEWESNGQPENNYKTTPPVLDSDGSFFLYSKLTVDKSRWQQGNVFSCSVMHEALHNHYTQKSLSLSPGKGGSDYKDDDDK

SEQ ID NO: 63 - protein, 384 aa, synthetic construct
MEFGLSWLFLVAILKGVQCEVQLLESGGGLVQPGGSLRLSCAVSGFTFNSFAMSWVRQAPGKGLEWVSAISGSGGGTYYADSVKGRFTISRDNSKNTLYLQMNSLRAEDTAVYFCAKDKILWFGEPVFDYWGQGTLVTVSSGGGSGGGGSYVLTQPSSVSVAPGQTATISCGGHNIGSKNVHWYQQRPGQSPVLVIYQDNKRPSGIPERFSGSNSGNTATLTISGTQAMDEADYYCQVWDNYSVLFGGGTKLTVLGGGGSGGGGSGGGGSNWVNVISDLKKIEDLIQSMHIDATLYTESDVHPSCKVTAMKCFLLELQVISCESGDASIHDTVENLIILANNSLSSNGNVTESGCKECEELEEKNIKEFLQSFVHIVQMFINTS

SEQ ID NO: 64 - protein, 586 aa, synthetic construct
MDMRVPAQLLGLLLLWFPGSRCSYVLTQPSSVSVAPGQTATISCGGHNIGSKNVHWYQQRPGQSPVLVIYQDNKRPSGIPERFSGSNSGNTATLTISGTQAMDEADYYCQVWDNYSVLFGGGTKLTVLGGGSGGGGEVQLLESGGGLVQPGGSLRLSCAVSGFTFNSFAMSWVRQAPGKGLEWVSAISGSGGGTYYADSVKGRFTISRDNSKNTLYLQMNSLRAEDTAVYFCAKDKILWFGEPVFDYWGQGTLVTVSSGGGGSGGGGSGGGGSITCPPPMSVEHADIWVKSYSLYSRERYICNSGFKRKAGTCSLTECVLNKATNVAHWTTPSLKCIRGGGGSEPKSSDKTHTCPPCPAPEAAGGPSVFLFPPKPKDTLMISRTPEVTCVVVDVSHEDPEVKFNWYVDGVEVHNAKTKPREEQYNSTYRVVSVLTVLHQDWLNGKEYKCKVSNKALPAPIEKTISKAKGQPREPQVYTLPPSRDELTKNQVSLWCLVKGFYPSDIAVEWESNGQPENNYKTTPPVLDSDGSFFLYSKLTVDKSRWQQGNVFSCSVMHEALHNHYTQKSLSLSPGKGGSDYKDDDDK

SEQ ID NO: 65 - protein, 386 aa, synthetic construct
MDMRVPAQLLGLLLLWFPGSRCEIVLTQSPATLSLSPGERATLSCRASQSVSSYLAWYQQKPGQAPRLLIYDASNRATGIPARFSGSGSGTDFTLTISSLEPEDFAVYYCQQRSNWPPTFGQGTKVEIKGGGSGGGGQVQLVQSGAEVKKPGESLKVSCKASGYTFTSYYMHWVRQAPGQGLEWMGIINPSGGSTSYAQKFQGRVTMTRDTSTSTVYMELSSLRSEDTAVYYCARGSAYYYDFADYWGQGTLVTVSSGGGGSGGGGSGGGGSNWVNVISDLKKIEDLIQSMHIDATLYTESDVHPSCKVTAMKCFLLELQVISCESGDASIHDTVENLIILANNSLSSNGNVTESGCKECEELEEKNIKEFLQSFVHIVQMFINTS

SEQ ID NO: 66 - protein, 585 aa, synthetic construct
MDMRVPAQLLGLLLLWFPGSRCEIVLTQSPATLSLSPGERATLSCRASQSVSSYLAWYQQKPGQAPRLLIYDASNRATGIPARFSGSGSGTDFTLTISSLEPEDFAVYYCQQRSNWPPTFGQGTKVEIKGGGSGGGGQVQLVQSGAEVKKPGESLKVSCKASGYTFTSYYMHWVRQAPGQGLEWMGIINPSGGSTSYAQKFQGRVTMTRDTSTSTVYMELSSLRSEDTAVYYCARGSAYYYDFADYWGQGTLVTVSSGGGGSGGGGSGGGGSITCPPPMSVEHADIWVKSYSLYSRERYICNSGFKRKAGTCSLTECVLNKATNVAHWTTPSLKCIRGGGGSEPKSSDKTHTCPPCPAPEAAGGPSVFLFPPKPKDTLMISRTPEVTCVVVDVSHEDPEVKFNWYVDGVEVHNAKTKPREEQYNSTYRVVSVLTVLHQDWLNGKEYKCKVSNKALPAPIEKTISKAKGQPREPQVYTLPPSRDELTKNQVSLWCLVKGFYPSDIAVEWESNGQPENNYKTTPPVLDSDGSFFLYSKLTVDKSRWQQGNVFSCSVMHEALHNHYTQKSLSLSPGKGGSDYKDDDDK

SEQ ID NO: 67 - protein, 387 aa, synthetic construct
MDMRVPAQLLGLLLLWFPGSRCSYVLTQPSSVSVAPGQTATISCGGHNIGSKNVHWYQQRPGQSPVLVIYQDNKRPSGIPERFSGSNSGNTATLTISGTQAMDEADYYCQVWDNYSVLFGGGTKLTVLGGGSGGGGEVQLLESGGGLVQPGGSLRLSCAVSGFTFNSFAMSWVRQAPGKGLEWVSAISGSGGGTYYADSVKGRFTISRDNSKNTLYLQMNSLRAEDTAVYFCAKDKILWFGEPVFDYWGQGTLVTVSSGGGGSGGGGSGGGGSNWVNVISDLKKIEDLIQSMHIDATLYTESDVHPSCKVTAMKCFLLELQVISCESGDASIHDTVENLIILANNSLSSNGNVTESGCKECEELEEKNIKEFLQSFVHIVQMFINTS

SEQ ID NO: 68 - protein, 377 aa, synthetic construct
MEFGLSWLFLVAILKGVQCQVQLVQSGAEVKKPGESVKVSCKASGYTFTNYGMNWVKQAPGQGLEWMGWINTYTGEPTYADKFQGRVTMTTDTSTSTAYMEIRNLGGDDTAVYYCARWSWSDGYYVYFDYWGQGTSVTVSSGGGSGGGGSYVLTQPSSVSVAPGQTATISCGGHNIGSKNVHWYQQRPGQSPVLVIYQDNKRPSGIPERFSGSNSGNTATLTISGTQAMDEADYYCQVWDNYSVLFGGGTKLTVLGGGGSGGGGSGGGGSRTVAAPSVFIFPPSDEQLKSGTASVVCLLNNFYPREAKVQWKVDNALQSGNSQESVTEQDSKDSTYSLSSTLTLSKADYEKHKVYACEVTHQGLSSPVTKSFNRGEC

SEQ ID NO: 69 - protein, 614 aa, synthetic construct
MEFGLSWLFLVAILKGVQCQVQLVQSGAEVKKPGESLKVSCKASGYTFTSYYMHWVRQAPGQGLEWMGIINPSGGSTSYAQKFQGRVTMTRDTSTSTVYMELSSLRSEDTAVYYCARGSAYYYDFADYWGQGTLVTVSSGGGSGGGGDIVMTQSPDSLTVSLGERTTINCKSSQSVLDSSTNKNSLAWYQQKPGQPPKLLLSWASTRESGIPDRFSGSGSGTDFTLTIDSPQPEDSATYYCQQSAHFPITFGQGTRLEIKGGGGSGGGGSGGGGSASTKGPSVFPLAPSSKSTSGGTAALGCLVKDYFPEPVTVSWNSGALTSGVHTFPAVLQSSGLYSLSSVVTVPSSSLGTQTYICNVNHKPSNTKVDKKVEPKSCDKTHTCPPCPAPEAAGGPSVFLFPPKPKDTLMISRTPEVTCVVVDVSHEDPEVKFNWYVDGVEVHNAKTKPREEQYNSTYRVVSVLTVLHQDWLNGKEYKCKVSNKALPAPIEKTISKAKGQPREPQVYTLPPSREEMTKNQVSLSCAVKGFYPSDIAVEWESNGQPENNYKTTPPVLDSDGSFFLVSKLTVDKSRWQQGNVFSCSVMHEALHNRYTQKSLSLSPGKGGSHHHHHH

SEQ ID NO: 70 - protein, 469 aa, synthetic construct; identical to SEQ ID NO: 9

SEQ ID NO: 71 - protein, 242 aa, synthetic construct; identical to SEQ ID NO: 10

SEQ ID NO: 72 - protein, 382 aa, synthetic construct
MEFGLSWLFLVAILKGVQCQVQLVQSGAEVKKPGESLKVSCKASGYTFTSYYMHWVRQAPGQGLEWMGIINPSGGSTSYAQKFQGRVTMTRDTSTSTVYMELSSLRSEDTAVYYCARGSAYYYDFADYWGQGTLVTVSSGGGSGGGGDIVMTQSPDSLTVSLGERTTINCKSSQSVLDSSTNKNSLAWYQQKPGQPPKLLLSWASTRESGIPDRFSGSGSGTDFTLTIDSPQPEDSATYYCQQSAHFPITFGQGTRLEIKGGGGSGGGGSGGGGSRTVAAPSVFIFPPSDEQLKSGTASVVCLLNNFYPREAKVQWKVDNALQSGNSQESVTEQDSKDSTYSLSSTLTLSKADYEKHKVYACEVTHQGLSSPVTKSFNRGEC

SEQ ID NO: 73 - protein, 600 aa, synthetic construct
MEFGLSWLFLVAILKGVQCQVQLVQSGAEVKKPGESVKVSCKASGYTFTNYGMNWVKQAPGQGLEWMGWINTYTGEPTYADKFQGRVTMTTDTSTSTAYMEIRNLGGDDTAVYYCARWSWSDGYYVYFDYWGQGTSVTVSSGGGSGGGGSYVLTQPSSVSVAPGQTATISCGGHNIGSKNVHWYQQRPGQSPVLVIYQDNKRPSGIPERFSGSNSGNTATLTISGTQAMDEADYYCQVWDNYSVLFGGGTKLTVLGGGGSGGGGSGGGGSASTKGPSVFPLAPSSKSTSGGTAALGCLVKDYFPEPVTVSWNSGALTSGVHTFPAVLQSSGLYSLSSVVTVPSSSLGTQTYICNVNHKPSNTKVDKKVEPKSCDKTHTCPPCPAPEAAGGPSVFLFPPKPKDTLMISRTPEVTCVVVDVSHEDPEVKFNWYVDGVEVHNAKTKPREEQYNSTYRVVSVLTVLHQDWLNGKEYKCKVSNKALPAPIEKTISKAKGQPREPQVYTLPPSREEMTKNQVSLSCAVKGFYPSDIAVEWESNGQPENNYKTTPPVLDSDGSFFLVSKLTVDKSRWQQGNVFSCSVMHEALHNRYTQKSLSLSPGK

SEQ ID NO: 74 - protein, 385 aa, synthetic construct
MDMRVPAQLLGLLLLWFPGSRCDIVMTQSPDSLTVSLGERTTINCKSSQSVLDSSTNKNSLAWYQQKPGQPPKLLLSWASTRESGIPDRFSGSGSGTDFTLTIDSPQPEDSATYYCQQSAHFPITFGQGTRLEIKGGGSGGGGQVQLVQSGAEVKKPGESLKVSCKASGYTFTSYYMHWVRQAPGQGLEWMGIINPSGGSTSYAQKFQGRVTMTRDTSTSTVYMELSSLRSEDTAVYYCARGSAYYYDFADYWGQGTLVTVSSGGGGSGGGGSGGGGSRTVAAPSVFIFPPSDEQLKSGTASVVCLLNNFYPREAKVQWKVDNALQSGNSQESVTEQDSKDSTYSLSSTLTLSKADYEKHKVYACEVTHQGLSSPVTKSFNRGEC

SEQ ID NO: 75 - protein, 612 aa, synthetic construct
MDMRVPAQLLGLLLLWFPGSRCSYVLTQPSSVSVAPGQTATISCGGHNIGSKNVHWYQQRPGQSPVLVIYQDNKRPSGIPERFSGSNSGNTATLTISGTQAMDEADYYCQVWDNYSVLFGGGTKLTVLGGGSGGGGQVQLVQSGAEVKKPGESVKVSCKASGYTFTNYGMNWVKQAPGQGLEWMGWINTYTGEPTYADKFQGRVTMTTDTSTSTAYMEIRNLGGDDTAVYYCARWSWSDGYYVYFDYWGQGTSVTVSSGGGGSGGGGSGGGGSASTKGPSVFPLAPSSKSTSGGTAALGCLVKDYFPEPVTVSWNSGALTSGVHTFPAVLQSSGLYSLSSVVTVPSSSLGTQTYICNVNHKPSNTKVDKKVEPKSCDKTHTCPPCPAPEAAGGPSVFLFPPKPKDTLMISRTPEVTCVVVDVSHEDPEVKFNWYVDGVEVHNAKTKPREEQYNSTYRVVSVLTVLHQDWLNGKEYKCKVSNKALPAPIEKTISKAKGQPREPQVYTLPPSREEMTKNQVSLSCAVKGFYPSDIAVEWESNGQPENNYKTTPPVLDSDGSFFLVSKLTVDKSRWQQGNVFSCSVMHEALHNRYTQKSLSLSPGKGGSHHHHHH

SEQ ID NO: 76 - protein, 380 aa, synthetic construct
MDMRVPAQLLGLLLLWFPGSRCSYVLTQPSSVSVAPGQTATISCGGHNIGSKNVHWYQQRPGQSPVLVIYQDNKRPSGIPERFSGSNSGNTATLTISGTQAMDEADYYCQVWDNYSVLFGGGTKLTVLGGGSGGGGQVQLVQSGAEVKKPGESVKVSCKASGYTFTNYGMNWVKQAPGQGLEWMGWINTYTGEPTYADKFQGRVTMTTDTSTSTAYMEIRNLGGDDTAVYYCARWSWSDGYYVYFDYWGQGTSVTVSSGGGGSGGGGSGGGGSRTVAAPSVFIFPPSDEQLKSGTASVVCLLNNFYPREAKVQWKVDNALQSGNSQESVTEQDSKDSTYSLSSTLTLSKADYEKHKVYACEVTHQGLSSPVTKSFNRGEC

SEQ ID NO: 77 - protein, 608 aa, synthetic construct
MDMRVPAQLLGLLLLWFPGSRCDIVMTQSPDSLTVSLGERTTINCKSSQSVLDSSTNKNSLAWYQQKPGQPPKLLLSWASTRESGIPDRFSGSGSGTDFTLTIDSPQPEDSATYYCQQSAHFPITFGQGTRLEIKGGGSGGGGQVQLVQSGAEVKKPGESLKVSCKASGYTFTSYYMHWVRQAPGQGLEWMGIINPSGGSTSYAQKFQGRVTMTRDTSTSTVYMELSSLRSEDTAVYYCARGSAYYYDFADYWGQGTLVTVSSGGGGSGGGGSGGGGSASTKGPSVFPLAPSSKSTSGGTAALGCLVKDYFPEPVTVSWNSGALTSGVHTFPAVLQSSGLYSLSSVVTVPSSSLGTQTYICNVNHKPSNTKVDKKVEPKSCDKTHTCPPCPAPEAAGGPSVFLFPPKPKDTLMISRTPEVTCVVVDVSHEDPEVKFNWYVDGVEVHNAKTKPREEQYNSTYRVVSVLTVLHQDWLNGKEYKCKVSNKALPAPIEKTISKAKGQPREPQVYTLPPSREEMTKNQVSLSCAVKGFYPSDIAVEWESNGQPENNYKTTPPVLDSDGSFFLVSKLTVDKSRWQQGNVFSCSVMHEALHNRYTQKSLSLSPGK

SEQ ID NO: 78 - protein, 338 aa, synthetic construct
DIVMTQSPDSLTVSLGERTTINCKSSQSVLDSSTNKNSLAWYQQKPGQPPKLLLSWASTRESGIPDRFSGSGSGTDFTLTIDSPQPEDSATYYCQQSAHFPITFGQGTRLEIKTVAAPSVFIFPPSYVLTQPSSVSVAPGQTATISCGGHNIGSKNVHWYQQRPGQSPVLVIYQDNKRPSGIPERFSGSNSGNTATLTISGTQAMDEADYYCQVWDNYSVLFGGGTKLTVLRTVAAPSVFIFPPSDEQLKSGTASVVCLLNNFYPREAKVQWKVDNALQSGNSQESVTEQDSKDSTYSLSSTLTLSKADYEKHKVYACEVTHQGLSSPVTKSFNRGEC

SEQ ID NO: 79 - protein, 587 aa, synthetic construct
QVQLVQSGAEVKKPGESVKVSCKASGYTFTNYGMNWVKQAPGQGLEWMGWINTYTGEPTYADKFQGRVTMTTDTSTSTAYMEIRNLGGDDTAVYYCARWSWSDGYYVYFDYWGQGTSVTVSSASTKGPQVQLVQSGAEVKKPGESLKVSCKASGYTFTSYYMHWVRQAPGQGLEWMGIINPSGGSTSYAQKFQGRVTMTRDTSTSTVYMELSSLRSEDTAVYYCARGSAYYYDFADYWGQGTLVTVSSASTKGPSVFPLAPSSKSTSGGTAALGCLVKDYFPEPVTVSWNSGALTSGVHTFPAVLQSSGLYSLSSVVTVPSSSLGTQTYICNVNHKPSNTKVDKKVEPKSCDKTHTCPPCPAPEAAGGPSVFLFPPKPKDTLMISRTPEVTCVVVDVSHEDPEVKFNWYVDGVEVHNAKTKPREEQYNSTYRVVSVLTVLHQDWLNGKEYKCKVSNKALPAPIEKTISKAKGQPREPQVYTLPPSREEMTKNQVSLSCAVKGFYPSDIAVEWESNGQPENNYKTTPPVLDSDGSFFLVSKLTVDKSRWQQGNVFSCSVMHEALHNRYTQKSLSLSPGKGGSHHHHHH

SEQ ID NO: 80 - protein, 442 aa, synthetic construct
MEFGLSWLFLVAILKGVQCSYVLTQPSSVSVAPGQTATISCGGHNIGSKNVHWYQQRPGQSPVLVIYQDNKRPSGIPERFSGSNSGNTATLTISGTQAMDEADYYCQVWDNYSVLFGGGTKLTVLGGGGSGGGGSGGGGSITCPPPMSVEHADIWVKSYSLYSRERYICNSGFKRKAGTCSLTECVLNKATNVAHWTTPSLKCIRGGGGSEPKSSDKTHTCPPCPAPEAAGGPSVFLFPPKPKDTLMISRTPEVTCVVVDVSHEDPEVKFNWYVDGVEVHNAKTKPREEQYNSTYRVVSVLTVLHQDWLNGKEYKCKVSNKALPAPIEKTISKAKGQPREPQVYTLPPSRDELTKNQVSLWCLVKGFYPSDIAVEWESNGQPENNYKTTPPVLDSDGSFFLYSKLTVDKSRWQQGNVFSCSVMHEALHNHYTQKSLSLSPGK

SEQ ID NO: 81 - protein, 257 aa, synthetic construct
MEFGLSWLFLVAILKGVQCNWVNVISDLKKIEDLIQSMHIDATLYTESDVHPSCKVTAMKCFLLELQVISCESGDASIHDTVENLIILANNSLSSNGNVTESGCKECEELEEKNIKEFLQSFVHIVQMFINTSGGGGQVQLVQSGAEVKKPGESLKVSCKASGYTFTSYYMHWVRQAPGQGLEWMGIINPSGGSTSYAQKFQGRVTMTRDTSTSTVYMELSSLRSEDTAVYYCARGSAYYYDFADYWGQGTLVTVSS

SEQ ID NO: 82 - protein, 467 aa, synthetic construct
MEFGLSWLFLVAILKGVQCQVQLVQSGAEVKKPGESLKVSCKASGYTFTSYYMHWVRQAPGQGLEWMGIINPSGGSTSYAQKFQGRVTMTRDTSTSTVYMELSSLRSEDTAVYYCARGSAYYYDFADYWGQGTLVTVSSGGGGSGGGGSGGGGSITCPPPMSVEHADIWVKSYSLYSRERYICNSGFKRKAGTCSLTECVLNKATNVAHWTTPSLKCIRGGGGSEPKSSDKTHTCPPCPAPEAAGGPSVFLFPPKPKDTLMISRTPEVTCVVVDVSHEDPEVKFNWYVDGVEVHNAKTKPREEQYNSTYRVVSVLTVLHQDWLNGKEYKCKVSNKALPAPIEKTISKAKGQPREPQVYTLPPSRDELTKNQVSLWCLVKGFYPSDIAVEWESNGQPENNYKTTPPVLDSDGSFFLYSKLTVDKSRWQQGNVFSCSVMHEALHNHYTQKSLSLSPGKGGSDYKDDDDK

SEQ ID NO: 83 - protein, 243 aa, synthetic construct
MEFGLSWLFLVAILKGVQCNWVNVISDLKKIEDLIQSMHIDATLYTESDVHPSCKVTAMKCFLLELQVISCESGDASIHDTVENLIILANNSLSSNGNVTESGCKECEELEEKNIKEFLQSFVHIVQMFINTSGGGGSYVLTQPSSVSVAPGQTATISCGGHNIGSKNVHWYQQRPGQSPVLVIYQDNKRPSGIPERFSGSNSGNTATLTISGTQAMDEADYYCQVWDNYSVLFGGGTKLTVL

SEQ ID NO: 84 - protein, 467 aa, synthetic construct
MEFGLSWLFLVAILKGVQCITCPPPMSVEHADIWVKSYSLYSRERYICNSGFKRKAGTCSLTECVLNKATNVAHWTTPSLKCIRGGGGSGGGGSGGGGSQVQLVQSGAEVKKPGESLKVSCKASGYTFTSYYMHWVRQAPGQGLEWMGIINPSGGSTSYAQKFQGRVTMTRDTSTSTVYMELSSLRSEDTAVYYCARGSAYYYDFADYWGQGTLVTVSSGGGGSEPKSSDKTHTCPPCPAPEAAGGPSVFLFPPKPKDTLMISRTPEVTCVVVDVSHEDPEVKFNWYVDGVEVHNAKTKPREEQYNSTYRVVSVLTVLHQDWLNGKEYKCKVSNKALPAPIEKTISKAKGQPREPQVYTLPPSRDELTKNQVSLWCLVKGFYPSDIAVEWESNGQPENNYKTTPPVLDSDGSFFLYSKLTVDKSRWQQGNVFSCSVMHEALHNHYTQKSLSLSPGKGGSDYKDDDDK

SEQ ID NO: 85 - protein, 243 aa, synthetic construct
MEFGLSWLFLVAILKGVQCSYVLTQPSSVSVAPGQTATISCGGHNIGSKNVHWYQQRPGQSPVLVIYQDNKRPSGIPERFSGSNSGNTATLTISGTQAMDEADYYCQVWDNYSVLFGGGTKLTVLGGGGNWVNVISDLKKIEDLIQSMHIDATLYTESDVHPSCKVTAMKCFLLELQVISCESGDASIHDTVENLIILANNSLSSNGNVTESGCKECEELEEKNIKEFLQSFVHIVQMFINTS

SEQ ID NO: 86 - protein, 453 aa, synthetic construct
MEFGLSWLFLVAILKGVQCITCPPPMSVEHADIWVKSYSLYSRERYICNSGFKRKAGTCSLTECVLNKATNVAHWTTPSLKCIRGGGGSGGGGSGGGGSSYVLTQPSSVSVAPGQTATISCGGHNIGSKNVHWYQQRPGQSPVLVIYQDNKRPSGIPERFSGSNSGNTATLTISGTQAMDEADYYCQVWDNYSVLFGGGTKLTVLGGGGSEPKSSDKTHTCPPCPAPEAAGGPSVFLFPPKPKDTLMISRTPEVTCVVVDVSHEDPEVKFNWYVDGVEVHNAKTKPREEQYNSTYRVVSVLTVLHQDWLNGKEYKCKVSNKALPAPIEKTISKAKGQPREPQVYTLPPSRDELTKNQVSLWCLVKGFYPSDIAVEWESNGQPENNYKTTPPVLDSDGSFFLYSKLTVDKSRWQQGNVFSCSVMHEALHNHYTQKSLSLSPGKGGSDYKDDDDK

SEQ ID NO: 87 - protein, 257 aa, synthetic construct
MEFGLSWLFLVAILKGVQCQVQLVQSGAEVKKPGESLKVSCKASGYTFTSYYMHWVRQAPGQGLEWMGIINPSGGSTSYAQKFQGRVTMTRDTSTSTVYMELSSLRSEDTAVYYCARGSAYYYDFADYWGQGTLVTVSSGGGGNWVNVISDLKKIEDLIQSMHIDATLYTESDVHPSCKVTAMKCFLLELQVISCESGDASIHDTVENLIILANNSLSSNGNVTESGCKECEELEEKNIKEFLQSFVHIVQMFINTS

SEQ ID NO: 88 - protein, 205 aa, synthetic construct
MEFGLSWLFLVAILKGVQCSYVLTQPSSVSVAPGQTATISCGGHNIGSKNVHWYQQRPGQSPVLVIYQDNKRPSGIPERFSGSNSGNTATLTISGTQAMDEADYYCQVWDNYSVLFGGGTKLTVLGGGGSGGGGSGGGGSITCPPPMSVEHADIWVKSYSLYSRERYICNSGFKRKAGTCSLTECVLNKATNVAHWTTPSLKCIR

SEQ ID NO: 89 - protein, 494 aa, synthetic construct
MEFGLSWLFLVAILKGVQCNWVNVISDLKKIEDLIQSMHIDATLYTESDVHPSCKVTAMKCFLLELQVISCESGDASIHDTVENLIILANNSLSSNGNVTESGCKECEELEEKNIKEFLQSFVHIVQMFINTSGGGGQVQLVQSGAEVKKPGESLKVSCKASGYTFTSYYMHWVRQAPGQGLEWMGIINPSGGSTSYAQKFQGRVTMTRDTSTSTVYMELSSLRSEDTAVYYCARGSAYYYDFADYWGQGTLVTVSSGGGGSEPKSSDKTHTCPPCPAPEAAGGPSVFLFPPKPKDTLMISRTPEVTCVVVDVSHEDPEVKFNWYVDGVEVHNAKTKPREEQYNSTYRVVSVLTVLHQDWLNGKEYKCKVSNKALPAPIEKTISKAKGQPREPQVYTLPPSRDELTKNQVSLWCLVKGFYPSDIAVEWESNGQPENNYKTTPPVLDSDGSFFLYSKLTVDKSRWQQGNVFSCSVMHEALHNHYTQKSLSLSPGK

SEQ ID NO: 90 - protein, 219 aa, synthetic construct
MEFGLSWLFLVAILKGVQCQVQLVQSGAEVKKPGESLKVSCKASGYTFTSYYMHWVRQAPGQGLEWMGIINPSGGSTSYAQKFQGRVTMTRDTSTSTVYMELSSLRSEDTAVYYCARGSAYYYDFADYWGQGTLVTVSSGGGGSGGGGSGGGGSITCPPPMSVEHADIWVKSYSLYSRERYICNSGFKRKAGTCSLTECVLNKATNVAHWTTPSLKCIR

SEQ ID NO: 91 - protein, 491 aa, synthetic construct
MEFGLSWLFLVAILKGVQCNWVNVISDLKKIEDLIQSMHIDATLYTESDVHPSCKVTAMKCFLLELQVISCESGDASIHDTVENLIILANNSLSSNGNVTESGCKECEELEEKNIKEFLQSFVHIVQMFINTSGGGGSYVLTQPSSVSVAPGQTATISCGGHNIGSKNVHWYQQRPGQSPVLVIYQDNKRPSGIPERFSGSNSGNTATLTISGTQAMDEADYYCQVWDNYSVLFGGGTKLTVLGGGGSEPKSSDKTHTCPPCPAPEAAGGPSVFLFPPKPKDTLMISRTPEVTCVVVDVSHEDPEVKFNWYVDGVEVHNAKTKPREEQYNSTYRVVSVLTVLHQDWLNGKEYKCKVSNKALPAPIEKTISKAKGQPREPQVYTLPPSRDELTKNQVSLWCLVKGFYPSDIAVEWESNGQPENNYKTTPPVLDSDGSFFLYSKLTVDKSRWQQGNVFSCSVMHEALHNHYTQKSLSLSPGKGGSDYKDDDDK

SEQ ID NO: 92 - protein, 219 aa, synthetic construct
MEFGLSWLFLVAILKGVQCITCPPPMSVEHADIWVKSYSLYSRERYICNSGFKRKAGTCSLTECVLNKATNVAHWTTPSLKCIRGGGGSGGGGSGGGGSQVQLVQSGAEVKKPGESLKVSCKASGYTFTSYYMHWVRQAPGQGLEWMGIINPSGGSTSYAQKFQGRVTMTRDTSTSTVYMELSSLRSEDTAVYYCARGSAYYYDFADYWGQGTLVTVSS

SEQ ID NO: 93 - protein, 486 aa, synthetic construct
MEFGLSWLFLVAILKGVQCSYVLTQPSSVSVAPGQTATISCGGHNIGSKNVHWYQQRPGQSPVLVIYQDNKRPSGIPERFSGSNSGNTATLTISGTQAMDEADYYCQVWDNYSVLFGGGTKLTVLGGGGNWVNVISDLKKIEDLIQSMHIDATLYTESDVHPSCKVTAMKCFLLELQVISCESGDASIHDTVENLIILANNSLSSNGNVTESGCKECEELEEKNIKEFLQSFVHIVQMFINTSEPKSSDKTHTCPPCPAPEAAGGPSVFLFPPKPKDTLMISRTPEVTCVVVDVSHEDPEVKFNWYVDGVEVHNAKTKPREEQYNSTYRVVSVLTVLHQDWLNGKEYKCKVSNKALPAPIEKTISKAKGQPREPQVYTLPPSRDELTKNQVSLWCLVKGFYPSDIAVEWESNGQPENNYKTTPPVLDSDGSFFLYSKLTVDKSRWQQGNVFSCSVMHEALHNHYTQKSLSLSPGKGGSDYKDDDDK

SEQ ID NO: 94 - protein, 203 aa, synthetic construct
MEFGLSWLFLVAILKGVQCITCPPPMSVEHADIWVKSYSLYSRERYICNSGFKRKAGTCSLTECVLNKATNVAHWTTPSLKCIRGGGSGGGGGGGGSSYVLTQPSSVSVAPGQTATISCGGHNIGSKNVHWYQQRPGQSPVLVIYQDNKRPSGIPERFSGSNSGNTATLTISGTQAMDEADYYCQVWDNYSVLFGGGTKLTVL

SEQ ID NO: 95 - protein, 500 aa, synthetic construct
MEFGLSWLFLVAILKGVQCQVQLVQSGAEVKKPGESLKVSCKASGYTFTSYYMHWVRQAPGQGLEWMGIINPSGGSTSYAQKFQGRVTMTRDTSTSTVYMELSSLRSEDTAVYYCARGSAYYYDFADYWGQGTLVTVSSGGGGNWVNVISDLKKIEDLIQSMHIDATLYTESDVHPSCKVTAMKCFLLELQVISCESGDASIHDTVENLIILANNSLSSNGNVTESGCKECEELEEKNIKEFLQSFVHIVQMFINTSEPKSSDKTHTCPPCPAPEAAGGPSVFLFPPKPKDTLMISRTPEVTCVVVDVSHEDPEVKFNWYVDGVEVHNAKTKPREEQYNSTYRVVSVLTVLHQDWLNGKEYKCKVSNKALPAPIEKTISKAKGQPREPQVYTLPPSRDELTKNQVSLWCLVKGFYPSDIAVEWESNGQPENNYKTTPPVLDSDGSFFLYSKLTVDKSRWQQGNVFSCSVMHEALHNHYTQKSLSLSPGKGGSDYKDDDDK

SEQ ID NO: 96 - protein, 106 aa, synthetic construct
SYVLTQPSSVSVAPGQTATISCGGHNIGSKNVHWYQQRPGQSPVLVIYQDNKRPSGIPERFSGSNSGNTATLTISGTQAMDEADYYCQVWDNYSVLFGGGTKLTVL

SEQ ID NO: 97 - protein, 120 aa, synthetic construct
QVQLVQSGAEVKKPGESLKVSCKASGYTFTSYYMHWVRQAPGQGLEWMGIINPSGGSTSYAQKFQGRVTMTRDTSTSTVYMELSSLRSEDTAVYYCARGSAYYYDFADYWGQGTLVTVSS

SEQ ID NO: 98 - protein, 107 aa, synthetic construct [sequence omitted]

SEQ ID NO: 99 - protein, 122 aa, synthetic construct [sequence omitted]

SEQ ID NO: 100 - protein, 107 aa, synthetic construct
DIQMTQSPSSLSASVGDRVTITCKASQDVGIAVAWYQQKPGKVPKLLIYWASTRHTGVPDRFSGSGSGTDFTLTISSLQPEDVATYYCQQYSSYPYTFGQGTKVEIK

SEQ ID NO: 101 - protein, 119 aa, synthetic construct
EVQLVESGGGLVQPGGSLRLSCAASGFDFSRYWMSWVRQAPGKGLEWIGEINPDSSTINYAPSLKDKFIISRDNAKNSLYLQMNSLRAEDTAVYYCARPDGNYWYFDVWGQGTLVTVSS

SEQ ID NO: 102 - protein, 113 aa, synthetic construct
DIVMTQSPDSLTVSLGERTTINCKSSQSVLDSSTNKNSLAWYQQKPGQPPKLLLSWASTRESGIPDRFSGSGSGTDFTLTIDSPQPEDSATYYCQQSAHFPITFGQGTRLEIK

SEQ ID NO: 103 - protein, 122 aa, synthetic construct
QVQLVQSGAEVKKPGESVKVSCKASGYTFTNYGMNWVKQAPGQGLEWMGWINTYTGEPTYADKFQGRVTMTTDTSTSTAYMEIRNLGGDDTAVYYCARWSWSDGYYVYFDYWGQGTSVTVSS

SEQ ID NO: 104 - protein, 114 aa, synthetic construct
NWVNVISDLKKIEDLIQSMHIDATLYTESDVHPSCKVTAMKCFLLELQVISLESGDASIHDTVENLIILANNSLSSNGNVTESGCKECEELEEKNIKEFLQSFVHIVQMFINTS

SEQ ID NO: 105 - protein, 114 aa, synthetic construct
NWVNVISDLKKIEDLIQSMHIDATLYTESDVHPSCKVTAMKCFLLELQVISCESGDASIHDTVENLIILANNSLSSNGNVTESGCKECEELEEKNIKEFLQSFVHIVQMFINTS

SEQ ID NO: 106 - protein, 175 aa, synthetic construct
ITCPPPMSVEHADIWVKSYSLYSRERYICNSGFKRKAGTSSLTECVLNKATNVAHWTTPSLKCIRDPALVHQRPAPPSTVTTAGVTPQPESLSPSGKEPAASSPSSNNTAATTAAIVPGSQLMPSKSPSTGTTEISSHESSHGTPSQTTAKNWELTASASHQPPGVYPQGHSDTT

SEQ ID NO: 107 - protein, 65 aa, synthetic construct
ITCPPPMSVEHADIWVKSYSLYSRERYICNSGFKRKAGTSSLTECVLNKATNVAHWTTPSLKCIR

SEQ ID NO: 108 - protein, 73 aa, synthetic construct
ITCPPPMSVEHADIWVKSYSLYSRERYICNSGFKRKAGTSSLTECVLNKATNVAHWTTPSLKCIRDPALVHQR

SEQ ID NO: 109 - protein, 77 aa, synthetic construct
ITCPPPMSVEHADIWVKSYSLYSRERYICNSGFKRKAGTSSLTECVLNKATNVAHWTTPSLKCIRDPALVHQRPAPP

SEQ ID NO: 110 - protein, 86 aa, synthetic construct
ITCPPPMSVEHADIWVKSYSLYSRERYICNSGFKRKAGTSSLTECVLNKATNVAHWTTPSLKCIRDPALVHQRPAPPSTVTTAGVT

SEQ ID NO: 111 - protein, 102 aa, synthetic construct
ITCPPPMSVEHADIWVKSYSLYSRERYICNSGFKRKAGTSSLTECVLNKATNVAHWTTPSLKCIRDPALVHQRPAPPSTVTTAGVTPQPESLSPSGKEPAAS

SEQ ID NO: 112 - protein, 65 aa, synthetic construct
ITCPPPMSVEHADIWVKSYSLYSRERYICNSGFKRKAGTCSLTECVLNKATNVAHWTTPSLKCIR